European Patent Specification EP 3 565 579 B9, published October 4, 2023. Title: A PD1-41BBL FUSION PROTEIN AND METHODS OF USE THEREOF. Applicant: KAHR Medical Ltd. TYKOCINSKI, Mark L SHANI, Noam GOZLAN, Yosi DRANITZKI ELHALEL, Michal BREMER, Edwin KAMINSKY, Ido. The sequence listing filed with the application follows.

SEQUENCE LISTING (18 sequences)

SEQ ID NO: 1 - protein, 356 aa, Artificial sequence
  Amino-acid sequence of the chimera protein (PD1- G -4-1BBL)
PGWFLDSPDRPWNPPTFSPALLVVTEGDNATFTCSFSNTSESFVLNWYRMSPSNQTDKLAAFPEDRSQPGQDCRFRVTQLPNGRDFHMSVVRARRNDSGTYLCGAISLAPKAQIKESLRAELRVTERRAEVPTAHPSPSPRPAGQFQTLVGACPWAVSGARASPGSAASPRLREGPELSPDDPAGLLDLRQGMFAQLVAQNVLLIDGPLSWYSDPGLAGVSLTGGLSYKEDTKELVVAKAGVYYVFFQLELRRVVAGEGSGSVSLALHLQPLRSAAGAAALALTVDLPPASSEARNSAFGFQGRLLHLSAGQRLGVHLHTEARARHAWQLTQGATVLGLFRVTPEIPAGLPSPRSE

SEQ ID NO: 2 - protein, 150 aa, homo sapiens [sequence omitted]

SEQ ID NO: 3 - protein, 205 aa, homo sapiens
ACPWAVSGARASPGSAASPRLREGPELSPDDPAGLLDLRQGMFAQLVAQNVLLIDGPLSWYSDPGLAGVSLTGGLSYKEDTKELVVAKAGVYYVFFQLELRRVVAGEGSGSVSLALHLQPLRSAAGAAALALTVDLPPASSEARNSAFGFQGRLLHLSAGQRLGVHLHTEARARHAWQLTQGATVLGLFRVTPEIPAGLPSPRSE

SEQ ID NO: 4 - protein, 355 aa, Artificial sequence
  Amino-acid sequence of the chimera protein (PD1- 4-1BBL, no linker)
PGWFLDSPDRPWNPPTFSPALLVVTEGDNATFTCSFSNTSESFVLNWYRMSPSNQTDKLAAFPEDRSQPGQDCRFRVTQLPNGRDFHMSVVRARRNDSGTYLCGAISLAPKAQIKESLRAELRVTERRAEVPTAHPSPSPRPAGQFQTLVACPWAVSGARASPGSAASPRLREGPELSPDDPAGLLDLRQGMFAQLVAQNVLLIDGPLSWYSDPGLAGVSLTGGLSYKEDTKELVVAKAGVYYVFFQLELRRVVAGEGSGSVSLALHLQPLRSAAGAAALALTVDLPPASSEARNSAFGFQGRLLHLSAGQRLGVHLHTEARARHAWQLTQGATVLGLFRVTPEIPAGLPSPRSE

SEQ ID NO: 5 - protein, 362 aa, Artificial sequence
  Amino-acid sequence of His-tagged PD1-41BBL
HHHHHHPGWFLDSPDRPWNPPTFSPALLVVTEGDNATFTCSFSNTSESFVLNWYRMSPSNQTDKLAAFPEDRSQPGQDCRFRVTQLPNGRDFHMSVVRARRNDSGTYLCGAISLAPKAQIKESLRAELRVTERRAEVPTAHPSPSPRPAGQFQTLVGACPWAVSGARASPGSAASPRLREGPELSPDDPAGLLDLRQGMFAQLVAQNVLLIDGPLSWYSDPGLAGVSLTGGLSYKEDTKELVVAKAGVYYVFFQLELRRVVAGEGSGSVSLALHLQPLRSAAGAAALALTVDLPPASSEARNSAFGFQGRLLHLSAGQRLGVHLHTEARARHAWQLTQGATVLGLFRVTPEIPAGLPSPRSE

SEQ ID NO: 6 - protein, 554 aa, Artificial sequence
  Amino-acid sequence of SIRP alpha 41BBL
HHHHHEEELQVIQPDKSVLVAAGETATLRCTATSLIPVGPIQWFRGAGPGRELIYNQKEGHFPRVTTVSDLTKRNNMDFSIRIGNITPADAGTYYCVKFRKGSPDDVEFKSGAGTELSVRAKPSAPVVSGPAARATPQHTVSFTCESHGFSPRDITLKWFKNGNELSDFQTNVDPVGESVSYSIHSTAKVVLTREDVHSQVICEVAHVTLQGDPLRGTANLSETIRVPPTLEVTQQPVRAENQVNVTCQVRKFYPQRLQLTWLENGNVSRTETASTVTENKDGTYNWMSWLLVNVSAHRDDVKLTCQVEHDGQPAVSKSHDLKVSAHPKEQGSNTAAENTGSNERNIYGACPWAVSGARASPGSAASPRLREGPELSPDDPAGLLDLRQGMFAQLVAQNVLLIDGPLSWYSDPGLAGVSLTGGLSYKEDTKELVVAKAGVYYVFFQLELRRVVAGEGSGSVSLALHLQPLRSAAGAAALALTVDLPPASSEARNSAFGFQGRLLHLSAGQRLGVHLHTEARARHAWQLTQGATVLGLFRVTPEIPAGLPSPRSE

SEQ ID NO: 7 - protein, 312 aa, Artificial sequence
  Amino-acid sequence of PD1-CD70
HHHHHHPGWFLDSPDRPWNPPTFSPALLVVTEGDNATFTCSFSNTSESFVLNWYRMSPSNQTDKLAAFPEDRSQPGQDCRFRVTQLPNGRDFHMSVVRARRNDSGTYLCGAISLAPKAQIKESLRAELRVTERRAEVPTAHPSPSPRPAGQFQTLVGQRFAQAQQQLPLESLGWDVAELQLNHTGPQQDPRLYWQGGPALGRSFLHGPELDKGQLRIHRDGIYMVHIQVTLAICSSTTASRHHPTTLAVGICSPASRSISLLRLSFHQGCTIASQRLTPLARGDTLCTNLTGTLLPSRNTDETFFGVQWVRP

SEQ ID NO: 8 - DNA, 1086 bp, Artificial sequence
  Nucleic-acid sequence of PD1-41BBL (with his tag)
caccatcatcaccaccatcctggctggtttctggacagccccgacagaccttggaaccctcctacattcagccccgctctgctggtggttaccgagggcgataatgccaccttcacctgtagcttcagcaacaccagcgagagcttcgtgctgaactggtacagaatgagccccagcaaccagaccgacaagctggccgcctttcctgaggatagatctcagcccggccaggactgccggttcagagttacacagctgcccaacggccgggacttccacatgtctgtcgtccgggccagaagaaacgacagcggcacatatctgtgcggcgccatttctctggcccctaaggctcagatcaaagagagcctgagagccgagctgagagtgacagaaagacgggccgaagtgcccacagctcacccttcaccttctccaagacctgccggccagtttcagacactcgtgggagcttgtccttgggccgtttctggcgctagagcctctcctggatctgccgcttctcccagactgagagagggacctgagctgagccctgatgatcctgctggactgctggatctgagacagggcatgtttgcccagctggtggcccagaatgtgctgctgattgatggccctctgtcctggtacagcgatcctggacttgctggcgttagcctgactggcggcctgagctacaaagaggacaccaaagaactggtggtggccaaggccggcgtgtactacgtgttctttcagctggaactgcggagagtggtggccggcgaaggatctggatctgtgtctctggctctgcatctgcagcctctgagatctgctgctggtgctgctgctctggccctgacagttgatctgcctcctgcctctagcgaggccagaaactccgcctttggcttccaaggcagactgctgcacctgagcgctggacagagactgggagtccatctgcacacagaagccagagctagacacgcctggcagctgacacaaggcgctacagtgctgggcctgttcagagtgacccctgagattccagccggcctgccatctcctagatctgag

SEQ ID NO: 9 - DNA, 1068 bp, Artificial sequence
  Nucleic-acid sequence of PD1-41BBL
cctggctggtttctggacagccccgacagaccttggaaccctcctacattcagccccgctctgctggtggttaccgagggcgataatgccaccttcacctgtagcttcagcaacaccagcgagagcttcgtgctgaactggtacagaatgagccccagcaaccagaccgacaagctggccgcctttcctgaggatagatctcagcccggccaggactgccggttcagagttacacagctgcccaacggccgggacttccacatgtctgtcgtccgggccagaagaaacgacagcggcacatatctgtgcggcgccatttctctggcccctaaggctcagatcaaagagagcctgagagccgagctgagagtgacagaaagacgggccgaagtgcccacagctcacccttcaccttctccaagacctgccggccagtttcagacactcgtgggagcttgtccttgggccgtttctggcgctagagcctctcctggatctgccgcttctcccagactgagagagggacctgagctgagccctgatgatcctgctggactgctggatctgagacagggcatgtttgcccagctggtggcccagaatgtgctgctgattgatggccctctgtcctggtacagcgatcctggacttgctggcgttagcctgactggcggcctgagctacaaagaggacaccaaagaactggtggtggccaaggccggcgtgtactacgtgttctttcagctggaactgcggagagtggtggccggcgaaggatctggatctgtgtctctggctctgcatctgcagcctctgagatctgctgctggtgctgctgctctggccctgacagttgatctgcctcctgcctctagcgaggccagaaactccgcctttggcttccaaggcagactgctgcacctgagcgctggacagagactgggagtccatctgcacacagaagccagagctagacacgcctggcagctgacacaaggcgctacagtgctgggcctgttcagagtgacccctgagattccagccggcctgccatctcctagatctgag

SEQ ID NO: 10 - protein, 288 aa, Artificial sequence
  Amino-acid sequence of full length PD1
MQIPQAPWPVVWAVLQLGWRPGWFLDSPDRPWNPPTFSPALLVVTEGDNATFTCSFSNTSESFVLNWYRMSPSNQTDKLAAFPEDRSQPGQDCRFRVTQLPNGRDFHMSVVRARRNDSGTYLCGAISLAPKAQIKESLRAELRVTERRAEVPTAHPSPSPRPAGQFQTLVVGVVGGLLGSLVLLVWVLAVICSRAARGTIGARRTGQPLKEDPSAVPVFSVDYGELDFQWREKTPEPPVPCVPEQTEYATIVFPSGMGTSSPARRGSADGPRSAQPLRPEDGHCSWPL

SEQ ID NO: 11 - DNA, 867 bp, Artificial sequence
  Nucleic-acid sequence of full length PD1
atgcagatcccacaggcgccctggccagtcgtctgggcggtgctacaactgggctggcggccaggatggttcttagactccccagacaggccctggaacccccccaccttctccccagccctgctcgtggtgaccgaaggggacaacgccaccttcacctgcagcttctccaacacatcggagagcttcgtgctaaactggtaccgcatgagccccagcaaccagacggacaagctggccgccttccccgaggaccgcagccagcccggccaggactgccgcttccgtgtcacacaactgcccaacgggcgtgacttccacatgagcgtggtcagggcccggcgcaatgacagcggcacctacctctgtggggccatctccctggcccccaaggcgcagatcaaagagagcctgcgggcagagctcagggtgacagagagaagggcagaagtgcccacagcccaccccagcccctcacccaggccagccggccagttccaaaccctggtggttggtgtcgtgggcggcctgctgggcagcctggtgctgctagtctgggtcctggccgtcatctgctcccgggccgcacgagggacaataggagccaggcgcaccggccagcccctgaaggaggacccctcagccgtgcctgtgttctctgtggactatggggagctggatttccagtggcgagagaagaccccggagccccccgtgccctgtgtccctgagcagacggagtatgccaccattgtctttcctagcggaatgggcacctcatcccccgcccgcaggggctcagctgacggccctcggagtgcccagccactgaggcctgaggatggacactgctcttggcccctctga

SEQ ID NO: 12 - DNA, 450 bp, Artificial sequence
  Nucleic-acid sequence encoding the extracellular domain of the human PD1 protein
ccaggatggttcttagactccccagacaggccctggaacccccccaccttctccccagccctgctcgtggtgaccgaaggggacaacgccaccttcacctgcagcttctccaacacatcggagagcttcgtgctaaactggtaccgcatgagccccagcaaccagacggacaagctggccgccttccccgaggaccgcagccagcccggccaggactgccgcttccgtgtcacacaactgcccaacgggcgtgacttccacatgagcgtggtcagggcccggcgcaatgacagcggcacctacctctgtggggccatctccctggcccccaaggcgcagatcaaagagagcctgcgggcagagctcagggtgacagagagaagggcagaagtgcccacagcccaccccagcccctcacccaggccagccggccagttccaaaccctggtg

SEQ ID NO: 13 - protein, 254 aa, Artificial sequence
  Amino-acid sequence of full length 41BBL
MEYASDASLDPEAPWPPAPRARACRVLPWALVAGLLLLLLLAAACAVFLACPWAVSGARASPGSAASPRLREGPELSPDDPAGLLDLRQGMFAQLVAQNVLLIDGPLSWYSDPGLAGVSLTGGLSYKEDTKELVVAKAGVYYVFFQLELRRVVAGEGSGSVSLALHLQPLRSAAGAAALALTVDLPPASSEARNSAFGFQGRLLHLSAGQRLGVHLHTEARARHAWQLTQGATVLGLFRVTPEIPAGLPSPRSE

SEQ ID NO: 14 - DNA, 765 bp, Artificial sequence
  Nucleic-acid sequence of full length 41BBL
atggaatacgcctctgacgcttcactggaccccgaagccccgtggcctcccgcgccccgcgctcgcgcctgccgcgtactgccttgggccctggtcgcggggctgctgctgctgctgctgctcgctgccgcctgcgccgtcttcctcgcctgcccctgggccgtgtccggggctcgcgcctcgcccggctccgcggccagcccgagactccgcgagggtcccgagctttcgcccgacgatcccgccggcctcttggacctgcggcagggcatgtttgcgcagctggtggcccaaaatgttctgctgatcgatgggcccctgagctggtacagtgacccaggcctggcaggcgtgtccctgacggggggcctgagctacaaagaggacacgaaggagctggtggtggccaaggctggagtctactatgtcttctttcaactagagctgcggcgcgtggtggccggcgagggctcaggctccgtttcacttgcgctgcacctgcagccactgcgctctgctgctggggccgccgccctggctttgaccgtggacctgccacccgcctcctccgaggctcggaactcggccttcggtttccagggccgcttgctgcacctgagtgccggccagcgcctgggcgtccatcttcacactgaggccagggcacgccatgcctggcagcttacccagggcgccacagtcttgggactcttccgggtgacccccgaaatcccagccggactcccttcaccgaggtcggaataa

SEQ ID NO: 15 - DNA, 615 bp, Artificial sequence
  Nucleic-acid sequence encoding  the extracellular domain of the human 41BBL
gcctgcccctgggccgtgtccggggctcgcgcctcgcccggctccgcggccagcccgagactccgcgagggtcccgagctttcgcccgacgatcccgccggcctcttggacctgcggcagggcatgtttgcgcagctggtggcccaaaatgttctgctgatcgatgggcccctgagctggtacagtgacccaggcctggcaggcgtgtccctgacggggggcctgagctacaaagaggacacgaaggagctggtggtggccaaggctggagtctactatgtcttctttcaactagagctgcggcgcgtggtggccggcgagggctcaggctccgtttcacttgcgctgcacctgcagccactgcgctctgctgctggggccgccgccctggctttgaccgtggacctgccacccgcctcctccgaggctcggaactcggccttcggtttccagggccgcttgctgcacctgagtgccggccagcgcctgggcgtccatcttcacactgaggccagggcacgccatgcctggcagcttacccagggcgccacagtcttgggactcttccgggtgacccccgaaatcccagccggactcccttcaccgaggtcggaa

SEQ ID NO: 16 - protein, 167 aa, Artificial sequence
  PD1 amino acid sequence
MQIPQAPWPVVWAVLQLGWRPGWFLDSPDRPWNPPTFSPALLVVTEGDNATFTCSFSNTSESFVLNWYRMSPSNQTDKLAAFPEDRSQPGQDCRFRVTQLPNGRDFHMSVVRARRNDSGTYLCGAISLAPKAQIKESLRAELRVTERRAEVPTAHPSPSPRPAGQFQ

SEQ ID NO: 17 - protein, 122 aa, Artificial sequence
  PD1 amino acid sequence
DSPDRPWNPPTFSPALLVVTEGDNATFTCSFSNTSESFVLNWYRMSPSNQTDKLAAFPEDRSQPGQDCRFRVTQLPNGRDFHMSVVRARRNDSGTYLCGAISLAPKAQIKESLRAELRVTER

SEQ ID NO: 18 - DNA, 1170 bp, Artificial sequence
  The cloning sequence of PD1-41BBL in the vector
gaattcccgccgccaccatgggctggtcctgcatcattctgtttctggtggccacagccaccggcgtgcactctcaccatcatcaccaccatcctggctggtttctggacagccccgacagaccttggaaccctcctacattcagccccgctctgctggtggttaccgagggcgataatgccaccttcacctgtagcttcagcaacaccagcgagagcttcgtgctgaactggtacagaatgagccccagcaaccagaccgacaagctggccgcctttcctgaggatagatctcagcccggccaggactgccggttcagagttacacagctgcccaacggccgggacttccacatgtctgtcgtccgggccagaagaaacgacagcggcacatatctgtgcggcgccatttctctggcccctaaggctcagatcaaagagagcctgagagccgagctgagagtgacagaaagacgggccgaagtgcccacagctcacccttcaccttctccaagacctgccggccagtttcagacactcgtgggagcttgtccttgggccgtttctggcgctagagcctctcctggatctgccgcttctcccagactgagagagggacctgagctgagccctgatgatcctgctggactgctggatctgagacagggcatgtttgcccagctggtggcccagaatgtgctgctgattgatggccctctgtcctggtacagcgatcctggacttgctggcgttagcctgactggcggcctgagctacaaagaggacaccaaagaactggtggtggccaaggccggcgtgtactacgtgttctttcagctggaactgcggagagtggtggccggcgaaggatctggatctgtgtctctggctctgcatctgcagcctctgagatctgctgctggtgctgctgctctggccctgacagttgatctgcctcctgcctctagcgaggccagaaactccgcctttggcttccaaggcagactgctgcacctgagcgctggacagagactgggagtccatctgcacacagaagccagagctagacacgcctggcagctgacacaaggcgctacagtgctgggcctgttcagagtgacccctgagattccagccggcctgccatctcctagatctgagtgataagctt